European Patent Specification EP 4 387 467 B1, published March 11, 2026. Title: SWEETENER BLEND COMPRISING THAUMATIN AND BRAZZEIN. Applicant: Nomad Bioscience GmbH. Application WO. The sequence listing filed with the application follows.

SEQUENCE LISTING (10 sequences)

SEQ ID NO: 1 - protein, 207 aa, Thaumatococcus daniellii
ATFEIVNRCSYTVWAAASKGDAALDAGGRQLNSGESWTINVEPGTNGGKIWARTDCYFDDSGSGICKTGDCGGLLRCKRFGRPPTTLAEFSLNQYGKDYIDISNIKGFNVPMNFSPTTRGCRGVRCAADIVGQCPAKLKAPGGGCNDACTVFQTSEYCCTTGKCGPTEYSRFFKRLCPDAFSYVLDKPTTVTCPGSSNYRVTFCPTA

SEQ ID NO: 2 - protein, 207 aa, Thaumatococcus daniellii
ATFEIVNRCSYTVWAAASKGDAALDAGGRQLNSGESWTINVEPGTKGGKIWARTDCYFDDSGRGICRTGDCGGLLQCKRFGRPPTTLAEFSLNQYGKDYIDISNIKGFNVPMDFSPTTRGCRGVRCAADIVGQCPAKLKAPGGGCNDACTVFQTSEYCCTTGKCGPTEYSRFFKRLCPDAFSYVLDKPTTVTCPGSSNYRVTFCPTA

SEQ ID NO: 3 - protein, 207 aa, Thaumatococcus daniellii
ATFEIVNRCSYTVWAAASKGDAALDAGGRQLNSGESWTINVEPGTNGGKIWARTDCYFDDSGSGICKTGDCGGLLRCKRFGRPPTTLAEFSLNQYGKDYIDISNIKGFNVPMDFSPTTRGCRGVRCAADIVGQCPAKLKAPGGGCNDACTVFQTSEYCCTTGKCGPTEYSRFFKRLCPDAFSYVLDKPTTVTCPGSSNYRVTFCPTA

SEQ ID NO: 4 - protein, 207 aa, Thaumatococcus daniellii
ATFEIVNRCSYTVWAAASKGDAALDAGGRQLNSGESWTINVEPGTKGGKIWARTDCYFDDSGSGICKTGDCGGLLRCKRFGRPPTTLAEFSLNQYGKDYIDISNIKGFNVPMDFSPTTRGCRGVRCAADIVGQCPAKLKAPGGGCNDACTVFQTSEYCCTTGKCGPTEYSRFFKRLCPDAFSYVLDKPTTVTCPGSSNYRVTFCPTA

SEQ ID NO: 5 - protein, 53 aa, Pentadiplandra brazzeana
  MOD_RES 1: note = pyroglutamic acid
EDKCKKVYENYPVSKCQLANQCNYDCKLDKHARSGECFYDEKRNLQCICDYCE

SEQ ID NO: 6 - protein, 53 aa, Pentadiplandra brazzeana
DKCKKVYENYPVSKCQLANQCNYDCKLDKHARSGECFYDEKRNLQCICDYCEY

SEQ ID NO: 7 - protein, 54 aa, Pentadiplandra brazzeana
QDKCKKVYENYPVSKCQLANQCNYDCKLDKHARSGECFYDEKRNLQCICDYCEY

SEQ ID NO: 8 - DNA, 162 bp, Pentadiplandra brazzeana
  source 1..162: mol_type = other DNA
gacaagtgcaagaaggtctacgagaactacccggtgtccaagtgccagctggccaaccagtgcaactacgactgcaagctggacaagcacgcccgctccggcgagtgcttctacgacgagaagcgcaacctgcagtgcatctgcgactactgcgagtactaa

SEQ ID NO: 9 - DNA, 240 bp, synthetic construct
  source 1..240: mol_type = other DNA
atggggaagcaaatggccgccctgtgtggctttctcctcgtggcgttgctctggctcacgcccgacgtcgcgtcaggtgacaagtgcaagaaggtctacgagaactacccggtgtccaagtgccagctggccaaccagtgcaactacgactgcaagctggacaagcacgcccgctccggcgagtgcttctacgacgagaagcgcaacctgcagtgcatctgcgactactgcgagtactaa

SEQ ID NO: 10 - DNA, 9418 bp, synthetic construct
  source 1..9418: mol_type = other DNA
cctgtggttggcacatacaaatggacgaacggataaaccttttcacgcccttttaaatatccgattattctaataaacgctcttttctcttaggtttacccgccaatatatcctgtcaaacactgatagtttaaactgaaggcgggaaacgacaatctgatctaagctagcttggaattggtaccacgcgtttcgacaaaatttagaacgaacttaattatgatctcaaatacattgatacatatctcatctagatctaggttatcattatgtaagaaagttttgacgaatatggcacgacaaaatggctagactcgatgtaattggtatctcaactcaacattatacttataccaaacattagttagacaaaatttaaacaactattttttatgtatgcaagagtcagcatatgtataattgattcagaatcgttttgacgagttcggatgtagtagtagccattatttaatgtacatactaatcgtgaatagtgaatatgatgaaacattgtatcttattgtataaatatccataaacacatcatgaaagacactttctttcacggtctgaattaattatgatacaattctaatagaaaacgaattaaattacgttgaattgtatgaaatctaattgaacaagccaaccacgacgacgactaacgttgcctggattgactcggtttaagttaaccactaaaaaaacggagctgtcatgtaacacgcggatcgagcaggtcacagtcatgaagccatcaaagcaaaagaactaatccaagggctgagatgattaattagtttaaaaattagttaacacgagggaaaaggctgtctgacagccaggtcacgttatctttacctgtggtcgaaatgattcgtgtctgtcgattttaattatttttttgaaaggccgaaaataaagttgtaagagataaacccgcctatataaattcatatattttcctctccgctttgaagttttagttttattgcaacaacaacaacaaattacaataacaacaaacaaaatacaaacaacaacaacatggcacaatttcaacaaacaattgacatgcaaactctccaagccgctgcgggacgcaacagcttggtgaatgatttggcatctcgtcgcgtttacgataatgcagtcgaggagctgaatgctcgttccagacgtcccaaggtaataggaactttctggatctactttatttgctggatctcgatcttgttttctcaatttccttgagatctggaattcgtttaatttggatctgtgaacctccactaaatcttttggttttactagaatcgatctaagttgaccgatcagttagctcgattatagctaccagaatttggcttgaccttgatggagagatccatgttcatgttacctgggaaatgatttgtatatgtgaattgaaatctgaactgttgaagttagattgaatctgaacactgtcaatgttagattgaatctgaacactgtttaaggttagatgaagtttgtgtatagattcttcgaaactttaggatttgtagtgtcgtacgttgaacagaaagctatttctgattcaatcagggtttatttgactgtattgaactctttttgtgtgtttgcaggtccacttctccaaggcagtgtctacggaacagaccctgattgcaacaaacgcatatccggagttcgagatttcctttactcatacgcaatccgctgtgcactccttggccggaggccttcggtcacttgagttggagtatctcatgatgcaagttccgttcggttctctgacgtacgacatcggcggtaacttttccgcgcaccttttcaaagggcgcgattacgttcactgctgcatgcctaatctggatgtacgtgacattgctcgccatgaaggacacaaggaagctatttacagttatgtgaatcgtttgaaaaggcagcagcgtcctgtgcctgaataccagagggcagctttcaacaactacgctgagaacccgcacttcgtccattgcgacaaacctttccaacagtgtgaattgacgacagcgaatggcactgacacctacgctgtagctctccatagcatttatgatatccctgttgaggagttcggttctgcgctactcaggaagaatgtgaaaacttgtttcgcggcctttcatttccatgagaatatgcttctagattgtgatacagtcacactcgatgagattggagctacgttccagaaatcaggtaacattccttagttacctttcttttctttttccatcataagtttatagattgtacatgctttgagatttttctttgcaaacaatctcaggtgataacctgagcttcttcttccataatgagagcactctcaattacacccacagcttcagcaacatcatcaagtacgtgtgcaagacgttcttccctgctagtcaacgcttcgtgtaccacaaggagttcctggtcactagagtcaacacttggtactgcaagttcacgagagtggatacgttcactctgttccgtggtgtgtaccacaacaatgtggattgcgaagagttttacaaggctatggacgatgcgtggcactacaaaaagacgttagcaatgcttaatgccgagaggaccatcttcaaggataacgctgcgttaaacttctggttcccgaaggtgctcttgaaattggaagtcttcttttgttgtctaaacctatcaatttctttgcggaaatttatttgaagctgtagagttaaaattgagtcttttaaacttttgtaggtgagagacatggttatcgtccctctctttgacgcttctatcacaactggtaggatgtctaggagagaggttatggtgaacaaggacttcgtctacacggtcctaaatcacatcaagacctatcaagctaaggcactgacgtacgcaaacgtgctgagcttcgtggagtctattaggtctagagtgataattaacggtgtcactgccaggtaagttgttacttatgattgttttcctctctgctacatgtattttgttgttcatttctgtaagatataagaattgagttttcctctgatgatattattaggtctgaatgggacacagacaaggcaattctaggtccattagcaatgacattcttcctgatcacgaagctgggtcatgtgcaagatgaaataatcctgaaaaagttccagaagttcgacagaaccaccaatgagctgatttggacaagtctctgcgatgccctgatgggggttattccctcggtcaaggagacgcttgtgcgcggtggttttgtgaaagtagcagaacaagccttagagatcaaggttagtatcatatgaagaaatacctagtttcagttgatgaatgctattttctgacctcagttgttctcttttgagaattatttcttttctaatttgcctgatttttctattaattcattaggttcccgagctatactgtaccttcgccgaccgattggtactacagtacaagaaggcggaggagttccaatcgtgtgatctttccaaacctctagaagagtcagagaagtactacaacgcattatccgagctatcagtgcttgagaatctcgactcttttgacttagaggcgtttaagactttatgtcagcagaagaatgtggacccggatatggcagcaaaggtaaatcctggtccacacttttacgataaaaacacaagattttaaactatgaactgatcaataatcattcctaaaagaccacacttttgttttgtttctaaagtaatttttactgttataacaggtggtcgtagcaatcatgaagtcagaattgacgttgcctttcaagaaacctacagaagaggaaatctcggagtcgctaaaaccaggagaggggtcgtgtgcagagcataaggaagtgttgagcttacaaaatgatgctccgttcccgtgtgtgaaaaatctagttgaaggttccgtgccggcgtatggaatgtgtcctaagggtggtggtttcgacaaattggatgtggacattgctgatttccatctcaagagtgtagatgcagttaaaaagggaactatgatgtctgcggtgtacacagggtctatcaaagttcaacaaatgaagaactacatagattacttaagtgcgtcgctggcagctacagtctcaaacctctgcaaggtaagaggtcaaaaggtttccgcaatgatccctctttttttgtttctctagtttcaagaatttgggtatatgactaacttctgagtgttccttgatgcatatttgtgatgagacaaatgtttgttctatgttttaggtgcttagagatgttcacggcgttgacccagagtcacaggagaaatctggagtgtgggatgttaggagaggacgttggttacttaaacctaatgcgaaaagtcacgcgtggggtgtggcagaagacgccaaccacaagttggttattgtgttactcaactgggatgacggaaagccggtttgtgatgagacatggttcagggtggcggtgtcaagcgattccttgatatattcggatatgggaaaacttaagacgctcacgtcttgcagtccaaatggtgagccaccggagcctaacgccaaagtaattttggtcgatggtgttcccggttgtggaaaaacgaaggagattatcgaaaaggtaagttctgcatttggttatgctccttgcattttaggtgttcgtcgctcttccatttccatgaatagctaagattttttttctctgcattcattcttcttgcctcagttctaactgtttgtggtatttttgttttaattattgctacaggtaaacttctctgaagacttgattttagtccctgggaaggaagcttctaagatgatcatccggagggccaaccaagctggtgtgataagagcggataaggacaatgttagaacggtggattccttcttgatgcatccttctagaagggtgtttaagaggttgtttatcgatgaaggactaatgctgcatacaggttgtgtaaatttcctactgctgctatctcaatgtgacgtcgcatatgtgtatggggacacaaagcaaattccgttcatttgcagagtcgcgaactttccgtatccagcgcattttgcaaaactcgtcgctgatgagaaggaagtcagaagagttacgctcaggtaaagcaactgtgttttaatcaatttcttgtcaggatatatggattataacttaatttttgagaaatctgtagtatttggcgtgaaatgagtttgctttttggtttctcccgtgttataggtgcccggctgatgttacgtatttccttaacaagaagtatgacggggcggtgatgtgtaccagcgcggtagagagatccgtgaaggcagaagtggtgagaggaaagggtgcattgaacccaataaccttaccgttggagggtaaaattttgaccttcacacaagctgacaagttcgagttactggagaagggttacaaggtaaagtttccaactttcctttaccatatcaaactaaagttcgaaactttttatttgatcaacttcaaggccacccgatctttctattcctgattaatttgtgatgaatccatattgacttttgatggttacgcaggatgtgaacactgtgcacgaggtgcaaggggagacgtacgagaagactgctattgtgcgcttgacatcaactccgttagagatcatatcgagtgcgtcacctcatgttttggtggcgctgacaagacacacaacgtgttgtaaatattacaccgttgtgttggacccgatggtgaatgtgatttcagaaatggagaagttgtccaatttccttcttgacatgtatagagttgaagcaggtctgtctttcctatttcatatgtttaatcctaggaatttgatcaattgattgtatgtatgtcgatcccaagactttcttgttcacttatatcttaactctctctttgctgtttcttgcaggtgtccaatagcaattacaaatcgatgcagtattcaggggacagaacttgtttgttcagacgcccaagtcaggagattggcgagatatgcaattttactatgacgctcttcttcccggaaacagtactattctcaatgaatttgatgctgttacgatgaatttgagggatatttccttaaacgtcaaagattgcagaatcgacttctccaaatccgtgcaacttcctaaagaacaacctattttcctcaagcctaaaataagaactgcggcagaaatgccgagaactgcaggtaaaatattggatgccagacgatattctttcttttgatttgtaactttttcctgtcaaggtcgataaattttattttttttggtaaaaggtcgataatttttttttggagccattatgtaattttcctaattaactgaaccaaaattatacaaaccaggtttgctggaaaatttggttgcaatgatcaaaagaaacatgaatgcgccggatttgacagggacaattgacattgaggatactgcatctctggtggttgaaaagttttgggattcgtatgttgacaaggaatttagtggaacgaacgaaatgaccatgacaagggagagcttctccaggtaaggacttctcatgaatattagtggcagattagtgttgttaaagtctttggttagataatcgatgcctcctaattgtccatgttttactggttttctacaattaaaggtggctttcgaaacaagagtcatctacagttggtcagttagcggactttaactttgtggatttgccggcagtagatgagtacaagcatatgatcaagagtcaaccaaagcaaaagttagacttgagtattcaagacgaatatcctgcattgcagacgatagtctaccattcgaaaaagatcaatgcgattttcggtccaatgttttcagaacttacgaggatgttactcgaaaggattgactcttcgaagtttctgttctacaccagaaagacacctgcacaaatagaggacttcttttctgacctagactcaacccaggcgatggaaattctggaactcgacatttcgaagtacgataagtcacaaaacgagttccattgtgctgtagagtacaagatctgggaaaagttaggaattgatgagtggctagctgaggtctggaaacaaggtgagttcctaagttccatttttttgtaatccttcaatgttattttaacttttcagatcaacatcaaaattaggttcaattttcatcaaccaaataatatttttcatgtatatataggtcacagaaaaacgaccttgaaagattatacggccggaatcaaaacatgtctttggtatcaaaggaaaagtggtgatgtgacaacctttattggtaataccatcatcattgccgcatgtttgagctcaatgatccccatggacaaagtgataaaggcagctttttgtggagacgatagcctgatttacattcctaaaggtttagacttgcctgatattcaggcgggcgcgaacctcatgtggaacttcgaggccaaactcttcaggaagaagtatggttacttctgtggtcgttatgttattcaccatgatagaggagccattgtgtattacgatccgcttaaactaatatctaagttaggttgtaaacatattagagatgttgttcacttagaagagttacgcgagtctttgtgtgatgtagctagtaacttaaataattgtgcgtatttttcacagttagatgaggccgttgccgaggttcataagaccgcggtaggcggttcgtttgctttttgtagtataattaagtatttgtcagataagagattgtttagagatttgttctttgtttgataatgtcgatagtctcgtacgaacctaaggtgagtgatttcctcaatctttcgaagaaggaagagatcttgccgaaggctctaacgaggttaaaaaccgtgtctattagtactaaagatattatatctgtcaaggagtcggagactttgtgtgatatagatttgttaatcaatgtgccattagataagtatagatatgtgggtatcctaggagccgtttttaccggagagtggctagtgccagacttcgttaaaggtggagtgacgataagtgtgatagataagcgtctggtgaactcaaaggagtgcgtgattggtacgtacagagccgcagccaagagtaagaggttccagttcaaattggttccaaattactttgtgtccaccgtggacgcaaagaggaagccgtggcaggtaaggatttttatgatatagtatgcttatgtattttgtactgaaagcatatcctgcttcattgggatattactgaaagcatttaactacatgtaaactcacttgatgatcaataaacttgattttgcaggttcatgttcgtatacaagacttgaagattgaggcgggttggcagccgttagctctggaagtagtttcagttgctatggtcaccaataacgttgtcatgaagggtttgagggaaaaggtcgtcgcaataaatgatccggacgtcgaaggtttcgaaggtaagccatcttcctgcttatttttataatgaacatagaaataggaagttgtgcagagaaactaattaacctgactcaaaatctaccctcataattgttgtttgatattggtcttgtattttgcaggtgtggttgacgaattcgtcgattcggttgcagcatttaaagcggttgacaactttaaaagaaggaaaaagaaggttgaagaaaagggtgtagtaagtaagtataagtacagaccggagaagtacgccggtcctgattcgtttaatttgaaagaagaaaacgtcttacaacattacaaacccgaatcagtaccagtatttcgataagctagcaaacaagaaatggggaagcaaatggccgccctgtgtggctttctcctcgtggcgttgctctggctcacgcccgacgtcgcgtcaggtgacaagtgcaagaaggtctacgagaactacccggtgtccaagtgccagctggccaaccagtgcaactacgactgcaagctggacaagcacgcccgctccggcgagtgcttctacgacgagaagcgcaacctgcagtgcatctgcgactactgcgagtactaagcttactagagcgtggtgcgcacgatagcgcatagtgtttttctctccacttgaatcgaagagatagacttacggtgtaaatccgtaggggtggcgtaaaccaaattacgcaatgttttgggttccatttaaatcgaaaccccttatttcctggatcacctgttaacgcacgtttgacgtgtattacagtgggaataagtaaaagtgagaggttcgaatcctccctaaccccgggtagggg